European Patent Application EP 4 257 690 A2, published October 11, 2023. Title: CRISPR HYBRID DNA/RNA POLYNUCLEOTIDES AND METHODS OF USE. Applicant: CARIBOU BIOSCIENCES, INC. The sequence listing filed with the application follows.

SEQUENCE LISTING (254 sequences)

SEQ ID NO: 1 - RNA, 121 nt, synthetic construct
  misc_feature 1..121: note = Description of Artificial Sequence: Synthetic polynucleotide
  source 1..121: mol_type = other RNA
ggggccactagggacaggatgtctcagagctatgctgtcctggaaacaggacagcatagcaagttgagataaggctagtccgttatcaacttgaaaaagtggcaccgagtcggtgcttttt

SEQ ID NO: 2 - RNA, 73 nt, synthetic construct
  misc_feature 1..73: note = Description of Artificial Sequence: Synthetic oligonucleotide
  source 1..73: mol_type = other RNA
gcaggacagcatagcaagttgagataaggctagtccgttatcaacttgaaaaagtggcaccgagtcggtgctt

SEQ ID NO: 3 - DNA, 42 bp, synthetic construct
  misc_feature 1..42: note = Description of Artificial Sequence: Synthetic oligonucleotide
  source 1..42: mol_type = other DNA
gagtccgagcagaagaagaagtctcagagctatgctgtcctg

SEQ ID NO: 4 - DNA, 42 bp, synthetic construct
  misc_feature 1..42: note = Description of Artificial Sequence: Synthetic oligonucleotide
  source 1..42: mol_type = other DNA
gggtggggggagtttgctccgtctcagagctatgctgtcctg

SEQ ID NO: 5 - DNA, 42 bp, synthetic construct
  misc_feature 1..42: note = Description of Artificial Sequence: Synthetic oligonucleotide
  source 1..42: mol_type = other DNA
gtttgtgtttccataaactggtctcagagctatgctgtcctg

SEQ ID NO: 6 - DNA, 42 bp, synthetic construct
  misc_feature 1..42: note = Description of Artificial Sequence: Synthetic oligonucleotide
  source 1..42: mol_type = other DNA
tctgtgataacctcagtttagtctcagagctatgctgtcctg

SEQ ID NO: 7 - DNA, 42 bp, synthetic construct
  misc_feature 1..42: note = Description of Artificial Sequence: Synthetic oligonucleotide
  source 1..42: mol_type = other DNA
ggccactgtagtcctccagggtctcagagctatgctgtcctg

SEQ ID NO: 8 - DNA, 42 bp, synthetic construct
  misc_feature 1..42: note = Description of Artificial Sequence: Synthetic oligonucleotide
  source 1..42: mol_type = other DNA
gtcccccagccggtcagccagtctcagagctatgctgtcctg

SEQ ID NO: 9 - DNA, 42 bp, synthetic construct
  misc_feature 1..42: note = Description of Artificial Sequence: Synthetic oligonucleotide
  source 1..42: mol_type = other DNA
ggcagccagcatgatgagacgtctcagagctatgctgtcctg

SEQ ID NO: 10 - DNA, 42 bp, synthetic construct
  misc_feature 1..42: note = Description of Artificial Sequence: Synthetic oligonucleotide
  source 1..42: mol_type = other DNA
gaggagctccaagaagactggtctcagagctatgctgtcctg

SEQ ID NO: 11 - RNA, 42 nt, synthetic construct
  misc_feature 1..42: note = Description of Artificial Sequence: Synthetic oligonucleotide
  source 1..42: mol_type = other RNA
gagtccgagcagaagaagaagtctcagagctatgctgtcctg

SEQ ID NO: 12 - RNA, 42 nt, synthetic construct
  misc_feature 1..42: note = Description of Artificial Sequence: Synthetic oligonucleotide
  source 1..42: mol_type = other RNA
gggtggggggagtttgctccgtctcagagctatgctgtcctg

SEQ ID NO: 13 - RNA, 42 nt, synthetic construct
  misc_feature 1..42: note = Description of Artificial Sequence: Synthetic oligonucleotide
  source 1..42: mol_type = other RNA
gtttgtgtttccataaactggtctcagagctatgctgtcctg

SEQ ID NO: 14 - RNA, 42 nt, synthetic construct
  misc_feature 1..42: note = Description of Artificial Sequence: Synthetic oligonucleotide
  source 1..42: mol_type = other RNA
tctgtgataacctcagtttagtctcagagctatgctgtcctg

SEQ ID NO: 15 - RNA, 42 nt, synthetic construct
  misc_feature 1..42: note = Description of Artificial Sequence: Synthetic oligonucleotide
  source 1..42: mol_type = other RNA
ggccactgtagtcctccagggtctcagagctatgctgtcctg

SEQ ID NO: 16 - RNA, 42 nt, synthetic construct
  misc_feature 1..42: note = Description of Artificial Sequence: Synthetic oligonucleotide
  source 1..42: mol_type = other RNA
gtcccccagccggtcagccagtctcagagctatgctgtcctg

SEQ ID NO: 17 - RNA, 42 nt, synthetic construct
  misc_feature 1..42: note = Description of Artificial Sequence: Synthetic oligonucleotide
  source 1..42: mol_type = other RNA
ggcagccagcatgatgagacgtctcagagctatgctgtcctg

SEQ ID NO: 18 - RNA, 42 nt, synthetic construct
  misc_feature 1..42: note = Description of Artificial Sequence: Synthetic oligonucleotide
  source 1..42: mol_type = other RNA
gaggagctccaagaagactggtctcagagctatgctgtcctg

SEQ ID NO: 19 - RNA, 42 nt, synthetic construct; identical to SEQ ID NO: 11
  modified_base 4: mod_base = OTHER; note = thymine
  modified_base 31: mod_base = OTHER; note = thymine
  modified_base 33: mod_base = OTHER; note = thymine
  modified_base 36: mod_base = OTHER; note = thymine
  modified_base 38: mod_base = OTHER; note = thymine
  modified_base 41: mod_base = OTHER; note = thymine
  misc_feature 1..42: note = Description of Combined DNA/RNA Molecule: Synthetic oligonucleotide
  source 1..42: mol_type = other RNA

SEQ ID NO: 20 - RNA, 42 nt, synthetic construct; identical to SEQ ID NO: 12
  modified_base 4: mod_base = OTHER; note = thymine
  modified_base 13..14: mod_base = OTHER; note = thymine
  modified_base 31: mod_base = OTHER; note = thymine
  modified_base 33: mod_base = OTHER; note = thymine
  modified_base 36: mod_base = OTHER; note = thymine
  modified_base 38: mod_base = OTHER; note = thymine
  modified_base 41: mod_base = OTHER; note = thymine
  misc_feature 1..42: note = Description of Combined DNA/RNA Molecule: Synthetic oligonucleotide
  source 1..42: mol_type = other RNA

SEQ ID NO: 21 - RNA, 42 nt, synthetic construct; identical to SEQ ID NO: 13
  modified_base 2..4: mod_base = OTHER; note = thymine
  modified_base 6: mod_base = OTHER; note = thymine
  modified_base 8..10: mod_base = OTHER; note = thymine
  modified_base 14: mod_base = OTHER; note = thymine
  modified_base 31: mod_base = OTHER; note = thymine
  modified_base 33: mod_base = OTHER; note = thymine
  modified_base 36: mod_base = OTHER; note = thymine
  modified_base 38: mod_base = OTHER; note = thymine
  modified_base 41: mod_base = OTHER; note = thymine
  misc_feature 1..42: note = Description of Combined DNA/RNA Molecule: Synthetic oligonucleotide
  source 1..42: mol_type = other RNA

SEQ ID NO: 22 - RNA, 42 nt, synthetic construct; identical to SEQ ID NO: 14
  modified_base 1: mod_base = OTHER; note = thymine
  modified_base 3: mod_base = OTHER; note = thymine
  modified_base 5: mod_base = OTHER; note = thymine
  modified_base 8: mod_base = OTHER; note = thymine
  modified_base 13: mod_base = OTHER; note = thymine
  modified_base 31: mod_base = OTHER; note = thymine
  modified_base 33: mod_base = OTHER; note = thymine
  modified_base 36: mod_base = OTHER; note = thymine
  modified_base 38: mod_base = OTHER; note = thymine
  modified_base 41: mod_base = OTHER; note = thymine
  misc_feature 1..42: note = Description of Combined DNA/RNA Molecule: Synthetic oligonucleotide
  source 1..42: mol_type = other RNA

SEQ ID NO: 23 - RNA, 42 nt, synthetic construct; identical to SEQ ID NO: 15
  modified_base 7: mod_base = OTHER; note = thymine
  modified_base 9: mod_base = OTHER; note = thymine
  modified_base 12: mod_base = OTHER; note = thymine
  modified_base 31: mod_base = OTHER; note = thymine
  modified_base 33: mod_base = OTHER; note = thymine
  modified_base 36: mod_base = OTHER; note = thymine
  modified_base 38: mod_base = OTHER; note = thymine
  modified_base 41: mod_base = OTHER; note = thymine
  misc_feature 1..42: note = Description of Combined DNA/RNA Molecule: Synthetic oligonucleotide
  source 1..42: mol_type = other RNA

SEQ ID NO: 24 - RNA, 42 nt, synthetic construct; identical to SEQ ID NO: 16
  modified_base 2: mod_base = OTHER; note = thymine
  modified_base 14: mod_base = OTHER; note = thymine
  modified_base 31: mod_base = OTHER; note = thymine
  modified_base 33: mod_base = OTHER; note = thymine
  modified_base 36: mod_base = OTHER; note = thymine
  modified_base 38: mod_base = OTHER; note = thymine
  modified_base 41: mod_base = OTHER; note = thymine
  misc_feature 1..42: note = Description of Combined DNA/RNA Molecule: Synthetic oligonucleotide
  source 1..42: mol_type = other RNA

SEQ ID NO: 25 - RNA, 42 nt, synthetic construct; identical to SEQ ID NO: 17
  modified_base 12: mod_base = OTHER; note = thymine
  modified_base 31: mod_base = OTHER; note = thymine
  modified_base 33: mod_base = OTHER; note = thymine
  modified_base 36: mod_base = OTHER; note = thymine
  modified_base 38: mod_base = OTHER; note = thymine
  modified_base 41: mod_base = OTHER; note = thymine
  misc_feature 1..42: note = Description of Combined DNA/RNA Molecule: Synthetic oligonucleotide
  source 1..42: mol_type = other RNA

SEQ ID NO: 26 - RNA, 42 nt, synthetic construct; identical to SEQ ID NO: 18
  modified_base 8: mod_base = OTHER; note = thymine
  modified_base 31: mod_base = OTHER; note = thymine
  modified_base 33: mod_base = OTHER; note = thymine
  modified_base 36: mod_base = OTHER; note = thymine
  modified_base 38: mod_base = OTHER; note = thymine
  modified_base 41: mod_base = OTHER; note = thymine
  misc_feature 1..42: note = Description of Combined DNA/RNA Molecule: Synthetic oligonucleotide
  source 1..42: mol_type = other RNA

SEQ ID NO: 27 - DNA, 20 bp, Homo sapiens
  source 1..20: mol_type = genomic DNA
gagtccgagcagaagaagaa

SEQ ID NO: 28 - DNA, 20 bp, Homo sapiens
  source 1..20: mol_type = genomic DNA
gagttagagcagaagaagaa

SEQ ID NO: 29 - DNA, 20 bp, Homo sapiens
  source 1..20: mol_type = genomic DNA
aggtactagcagaagaagaa

SEQ ID NO: 30 - DNA, 20 bp, Homo sapiens
  source 1..20: mol_type = genomic DNA
acgtctgagcagaagaagaa

SEQ ID NO: 31 - DNA, 20 bp, Homo sapiens
  source 1..20: mol_type = genomic DNA
aggtgctagcagaagaagaa

SEQ ID NO: 32 - DNA, 20 bp, Homo sapiens
  source 1..20: mol_type = genomic DNA
gggtggggggagtttgctcc

SEQ ID NO: 33 - DNA, 20 bp, Homo sapiens
  source 1..20: mol_type = genomic DNA
ggatggagggagtttgctcc

SEQ ID NO: 34 - DNA, 20 bp, Homo sapiens
  source 1..20: mol_type = genomic DNA
ggggaggggaagtttgctcc

SEQ ID NO: 35 - DNA, 20 bp, Homo sapiens
  source 1..20: mol_type = genomic DNA
gggagggtggagtttgctcc

SEQ ID NO: 36 - DNA, 20 bp, Homo sapiens
  source 1..20: mol_type = genomic DNA
cgggggagggagtttgctcc

SEQ ID NO: 37 - DNA, 42 bp, synthetic construct
  misc_feature 1..42: note = Description of Artificial Sequence: Synthetic oligonucleotide
  source 1..42: mol_type = other DNA
ggggccactagggacaggatgtctcagagctatgctgtcctg

SEQ ID NO: 38 - RNA, 42 nt, synthetic construct
  modified_base 9: mod_base = OTHER; note = thymine
  modified_base 20: mod_base = OTHER; note = thymine
  modified_base 31: mod_base = OTHER; note = thymine
  modified_base 33: mod_base = OTHER; note = thymine
  modified_base 36: mod_base = OTHER; note = thymine
  modified_base 38: mod_base = OTHER; note = thymine
  modified_base 41: mod_base = OTHER; note = thymine
  misc_feature 1..42: note = Description of Combined DNA/RNA Molecule: Synthetic oligonucleotide
  source 1..42: mol_type = other RNA
ggggccactagggacaggatgtctcagagctatgctgtcctg

SEQ ID NO: 39 - RNA, 42 nt, synthetic construct; identical to SEQ ID NO: 38
  modified_base 9: mod_base = OTHER; note = thymine
  modified_base 20: mod_base = OTHER; note = thymine
  modified_base 22: mod_base = OTHER; note = thymine
  modified_base 24: mod_base = OTHER; note = thymine
  modified_base 31: mod_base = OTHER; note = thymine
  modified_base 33: mod_base = OTHER; note = thymine
  modified_base 36: mod_base = OTHER; note = thymine
  modified_base 38: mod_base = OTHER; note = thymine
  modified_base 41: mod_base = OTHER; note = thymine
  misc_feature 1..42: note = Description of Combined DNA/RNA Molecule: Synthetic oligonucleotide
  source 1..42: mol_type = other RNA

SEQ ID NO: 40 - RNA, 42 nt, synthetic construct; identical to SEQ ID NO: 38
  modified_base 9: mod_base = OTHER; note = thymine
  modified_base 22: mod_base = OTHER; note = thymine
  modified_base 24: mod_base = OTHER; note = thymine
  modified_base 31: mod_base = OTHER; note = thymine
  modified_base 33: mod_base = OTHER; note = thymine
  modified_base 36: mod_base = OTHER; note = thymine
  modified_base 38: mod_base = OTHER; note = thymine
  modified_base 41: mod_base = OTHER; note = thymine
  misc_feature 1..42: note = Description of Combined DNA/RNA Molecule: Synthetic oligonucleotide
  source 1..42: mol_type = other RNA

SEQ ID NO: 41 - RNA, 42 nt, synthetic construct; identical to SEQ ID NO: 38
  modified_base 9: mod_base = OTHER; note = thymine
  modified_base 31: mod_base = OTHER; note = thymine
  modified_base 33: mod_base = OTHER; note = thymine
  modified_base 36: mod_base = OTHER; note = thymine
  modified_base 38: mod_base = OTHER; note = thymine
  modified_base 41: mod_base = OTHER; note = thymine
  misc_feature 1..42: note = Description of Combined DNA/RNA Molecule: Synthetic oligonucleotide
  source 1..42: mol_type = other RNA

SEQ ID NO: 42 - RNA, 42 nt, synthetic construct; identical to SEQ ID NO: 38
  modified_base 22: mod_base = OTHER; note = thymine
  modified_base 24: mod_base = OTHER; note = thymine
  modified_base 31: mod_base = OTHER; note = thymine
  modified_base 33: mod_base = OTHER; note = thymine
  modified_base 36: mod_base = OTHER; note = thymine
  modified_base 38: mod_base = OTHER; note = thymine
  modified_base 41: mod_base = OTHER; note = thymine
  misc_feature 1..42: note = Description of Combined DNA/RNA Molecule: Synthetic oligonucleotide
  source 1..42: mol_type = other RNA

SEQ ID NO: 43 - RNA, 42 nt, synthetic construct; identical to SEQ ID NO: 38
  modified_base 9: mod_base = OTHER; note = thymine
  modified_base 20: mod_base = OTHER; note = thymine
  modified_base 31: mod_base = OTHER; note = thymine
  modified_base 33: mod_base = OTHER; note = thymine
  modified_base 36: mod_base = OTHER; note = thymine
  modified_base 38: mod_base = OTHER; note = thymine
  modified_base 41: mod_base = OTHER; note = thymine
  misc_feature 1..42: note = Description of Combined DNA/RNA Molecule: Synthetic oligonucleotide
  source 1..42: mol_type = other RNA

SEQ ID NO: 44 - RNA, 42 nt, synthetic construct; identical to SEQ ID NO: 38
  modified_base 9: mod_base = OTHER; note = thymine
  modified_base 22: mod_base = OTHER; note = thymine
  modified_base 24: mod_base = OTHER; note = thymine
  modified_base 31: mod_base = OTHER; note = thymine
  modified_base 33: mod_base = OTHER; note = thymine
  modified_base 36: mod_base = OTHER; note = thymine
  modified_base 38: mod_base = OTHER; note = thymine
  modified_base 41: mod_base = OTHER; note = thymine
  misc_feature 1..42: note = Description of Combined DNA/RNA Molecule: Synthetic oligonucleotide
  source 1..42: mol_type = other RNA

SEQ ID NO: 45 - RNA, 42 nt, synthetic construct; identical to SEQ ID NO: 38
  modified_base 9: mod_base = OTHER; note = thymine
  modified_base 20: mod_base = OTHER; note = thymine
  modified_base 31: mod_base = OTHER; note = thymine
  modified_base 33: mod_base = OTHER; note = thymine
  modified_base 36: mod_base = OTHER; note = thymine
  modified_base 38: mod_base = OTHER; note = thymine
  modified_base 41: mod_base = OTHER; note = thymine
  misc_feature 1..42: note = Description of Combined DNA/RNA Molecule: Synthetic oligonucleotide
  source 1..42: mol_type = other RNA

SEQ ID NO: 46 - RNA, 42 nt, synthetic construct; identical to SEQ ID NO: 38
  modified_base 22: mod_base = OTHER; note = thymine
  modified_base 24: mod_base = OTHER; note = thymine
  modified_base 31: mod_base = OTHER; note = thymine
  modified_base 33: mod_base = OTHER; note = thymine
  modified_base 36: mod_base = OTHER; note = thymine
  modified_base 38: mod_base = OTHER; note = thymine
  modified_base 41: mod_base = OTHER; note = thymine
  misc_feature 1..42: note = Description of Combined DNA/RNA Molecule: Synthetic oligonucleotide
  source 1..42: mol_type = other RNA

SEQ ID NO: 47 - RNA, 42 nt, synthetic construct; identical to SEQ ID NO: 38
  modified_base 20: mod_base = OTHER; note = thymine
  modified_base 31: mod_base = OTHER; note = thymine
  modified_base 33: mod_base = OTHER; note = thymine
  modified_base 36: mod_base = OTHER; note = thymine
  modified_base 38: mod_base = OTHER; note = thymine
  modified_base 41: mod_base = OTHER; note = thymine
  misc_feature 1..42: note = Description of Combined DNA/RNA Molecule: Synthetic oligonucleotide
  source 1..42: mol_type = other RNA

SEQ ID NO: 48 - RNA, 42 nt, synthetic construct; identical to SEQ ID NO: 38
  modified_base 20: mod_base = OTHER; note = thymine
  modified_base 31: mod_base = OTHER; note = thymine
  modified_base 33: mod_base = OTHER; note = thymine
  modified_base 36: mod_base = OTHER; note = thymine
  modified_base 38: mod_base = OTHER; note = thymine
  modified_base 41: mod_base = OTHER; note = thymine
  misc_feature 1..42: note = Description of Combined DNA/RNA Molecule: Synthetic oligonucleotide
  source 1..42: mol_type = other RNA

SEQ ID NO: 49 - RNA, 42 nt, synthetic construct; identical to SEQ ID NO: 38
  modified_base 9: mod_base = OTHER; note = thymine
  modified_base 22: mod_base = OTHER; note = thymine
  modified_base 31: mod_base = OTHER; note = thymine
  modified_base 33: mod_base = OTHER; note = thymine
  modified_base 36: mod_base = OTHER; note = thymine
  modified_base 38: mod_base = OTHER; note = thymine
  modified_base 41: mod_base = OTHER; note = thymine
  misc_feature 1..42: note = Description of Combined DNA/RNA Molecule: Synthetic oligonucleotide
  source 1..42: mol_type = other RNA

SEQ ID NO: 50 - RNA, 42 nt, synthetic construct; identical to SEQ ID NO: 38
  modified_base 9: mod_base = OTHER; note = thymine
  modified_base 24: mod_base = OTHER; note = thymine
  modified_base 31: mod_base = OTHER; note = thymine
  modified_base 33: mod_base = OTHER; note = thymine
  modified_base 36: mod_base = OTHER; note = thymine
  modified_base 38: mod_base = OTHER; note = thymine
  modified_base 41: mod_base = OTHER; note = thymine
  misc_feature 1..42: note = Description of Combined DNA/RNA Molecule: Synthetic oligonucleotide
  source 1..42: mol_type = other RNA

SEQ ID NO: 51 - RNA, 42 nt, synthetic construct; identical to SEQ ID NO: 38
  modified_base 9: mod_base = OTHER; note = thymine
  modified_base 20: mod_base = OTHER; note = thymine
  modified_base 22: mod_base = OTHER; note = thymine
  modified_base 24: mod_base = OTHER; note = thymine
  modified_base 31: mod_base = OTHER; note = thymine
  modified_base 33: mod_base = OTHER; note = thymine
  modified_base 36: mod_base = OTHER; note = thymine
  modified_base 38: mod_base = OTHER; note = thymine
  modified_base 41: mod_base = OTHER; note = thymine
  misc_feature 1..42: note = Description of Combined DNA/RNA Molecule: Synthetic oligonucleotide
  source 1..42: mol_type = other RNA

SEQ ID NO: 52 - RNA, 42 nt, synthetic construct; identical to SEQ ID NO: 38
  modified_base 9: mod_base = OTHER; note = thymine
  modified_base 22: mod_base = OTHER; note = thymine
  modified_base 24: mod_base = OTHER; note = thymine
  modified_base 31: mod_base = OTHER; note = thymine
  modified_base 33: mod_base = OTHER; note = thymine
  modified_base 36: mod_base = OTHER; note = thymine
  modified_base 38: mod_base = OTHER; note = thymine
  modified_base 41: mod_base = OTHER; note = thymine
  misc_feature 1..42: note = Description of Combined DNA/RNA Molecule: Synthetic oligonucleotide
  source 1..42: mol_type = other RNA

SEQ ID NO: 53 - RNA, 42 nt, synthetic construct; identical to SEQ ID NO: 38
  modified_base 9: mod_base = OTHER; note = thymine
  modified_base 20: mod_base = OTHER; note = thymine
  modified_base 24: mod_base = OTHER; note = thymine
  modified_base 31: mod_base = OTHER; note = thymine
  modified_base 33: mod_base = OTHER; note = thymine
  modified_base 36: mod_base = OTHER; note = thymine
  modified_base 38: mod_base = OTHER; note = thymine
  modified_base 41: mod_base = OTHER; note = thymine
  misc_feature 1..42: note = Description of Combined DNA/RNA Molecule: Synthetic oligonucleotide
  source 1..42: mol_type = other RNA

SEQ ID NO: 54 - RNA, 42 nt, synthetic construct; identical to SEQ ID NO: 38
  modified_base 9: mod_base = OTHER; note = thymine
  modified_base 20: mod_base = OTHER; note = thymine
  modified_base 22: mod_base = OTHER; note = thymine
  modified_base 31: mod_base = OTHER; note = thymine
  modified_base 33: mod_base = OTHER; note = thymine
  modified_base 36: mod_base = OTHER; note = thymine
  modified_base 38: mod_base = OTHER; note = thymine
  modified_base 41: mod_base = OTHER; note = thymine
  misc_feature 1..42: note = Description of Combined DNA/RNA Molecule: Synthetic oligonucleotide
  source 1..42: mol_type = other RNA

SEQ ID NO: 55 - RNA, 42 nt, synthetic construct; identical to SEQ ID NO: 38
  modified_base 9: mod_base = OTHER; note = thymine
  modified_base 20: mod_base = OTHER; note = thymine
  modified_base 22: mod_base = OTHER; note = thymine
  modified_base 24: mod_base = OTHER; note = thymine
  modified_base 31: mod_base = OTHER; note = thymine
  modified_base 33: mod_base = OTHER; note = thymine
  modified_base 36: mod_base = OTHER; note = thymine
  modified_base 38: mod_base = OTHER; note = thymine
  modified_base 41: mod_base = OTHER; note = thymine
  misc_feature 1..42: note = Description of Combined DNA/RNA Molecule: Synthetic oligonucleotide
  source 1..42: mol_type = other RNA

SEQ ID NO: 56 - RNA, 42 nt, synthetic construct; identical to SEQ ID NO: 38
  modified_base 9: mod_base = OTHER; note = thymine
  modified_base 20: mod_base = OTHER; note = thymine
  modified_base 24: mod_base = OTHER; note = thymine
  modified_base 31: mod_base = OTHER; note = thymine
  modified_base 33: mod_base = OTHER; note = thymine
  modified_base 36: mod_base = OTHER; note = thymine
  modified_base 38: mod_base = OTHER; note = thymine
  modified_base 41: mod_base = OTHER; note = thymine
  misc_feature 1..42: note = Description of Combined DNA/RNA Molecule: Synthetic oligonucleotide
  source 1..42: mol_type = other RNA

SEQ ID NO: 57 - RNA, 42 nt, synthetic construct; identical to SEQ ID NO: 38
  modified_base 9: mod_base = OTHER; note = thymine
  modified_base 20: mod_base = OTHER; note = thymine
  modified_base 22: mod_base = OTHER; note = thymine
  modified_base 31: mod_base = OTHER; note = thymine
  modified_base 33: mod_base = OTHER; note = thymine
  modified_base 36: mod_base = OTHER; note = thymine
  modified_base 38: mod_base = OTHER; note = thymine
  modified_base 41: mod_base = OTHER; note = thymine
  misc_feature 1..42: note = Description of Combined DNA/RNA Molecule: Synthetic oligonucleotide
  source 1..42: mol_type = other RNA

SEQ ID NO: 58 - RNA, 42 nt, synthetic construct; identical to SEQ ID NO: 38
  modified_base 9: mod_base = OTHER; note = thymine
  modified_base 20: mod_base = OTHER; note = thymine
  modified_base 22: mod_base = OTHER; note = thymine
  modified_base 24: mod_base = OTHER; note = thymine
  modified_base 31: mod_base = OTHER; note = thymine
  modified_base 33: mod_base = OTHER; note = thymine
  modified_base 36: mod_base = OTHER; note = thymine
  modified_base 38: mod_base = OTHER; note = thymine
  modified_base 41: mod_base = OTHER; note = thymine
  misc_feature 1..42: note = Description of Combined DNA/RNA Molecule: Synthetic oligonucleotide
  source 1..42: mol_type = other RNA

SEQ ID NO: 59 - RNA, 42 nt, synthetic construct; identical to SEQ ID NO: 38
  modified_base 9: mod_base = OTHER; note = thymine
  modified_base 20: mod_base = OTHER; note = thymine
  modified_base 22: mod_base = OTHER; note = thymine
  modified_base 24: mod_base = OTHER; note = thymine
  modified_base 31: mod_base = OTHER; note = thymine
  modified_base 33: mod_base = OTHER; note = thymine
  modified_base 36: mod_base = OTHER; note = thymine
  modified_base 38: mod_base = OTHER; note = thymine
  modified_base 41: mod_base = OTHER; note = thymine
  misc_feature 1..42: note = Description of Combined DNA/RNA Molecule: Synthetic oligonucleotide
  source 1..42: mol_type = other RNA

SEQ ID NO: 60 - DNA, 42 bp, synthetic construct; identical to SEQ ID NO: 37
  misc_feature 1..42: note = Description of Artificial Sequence: Synthetic oligonucleotide
  source 1..42: mol_type = other DNA

SEQ ID NO: 61 - RNA, 42 nt, synthetic construct; identical to SEQ ID NO: 38
  modified_base 9: mod_base = OTHER; note = thymine
  modified_base 20: mod_base = OTHER; note = thymine
  modified_base 22: mod_base = OTHER; note = thymine
  modified_base 24: mod_base = OTHER; note = thymine
  modified_base 31: mod_base = OTHER; note = thymine
  modified_base 33: mod_base = OTHER; note = thymine
  modified_base 36: mod_base = OTHER; note = thymine
  modified_base 38: mod_base = OTHER; note = thymine
  modified_base 41: mod_base = OTHER; note = thymine
  misc_feature 1..42: note = Description of Combined DNA/RNA Molecule: Synthetic oligonucleotide
  source 1..42: mol_type = other RNA

SEQ ID NO: 62 - RNA, 42 nt, synthetic construct; identical to SEQ ID NO: 38
  modified_base 9: mod_base = OTHER; note = thymine
  modified_base 20: mod_base = OTHER; note = thymine
  modified_base 22: mod_base = OTHER; note = thymine
  modified_base 24: mod_base = OTHER; note = thymine
  modified_base 31: mod_base = OTHER; note = thymine
  modified_base 33: mod_base = OTHER; note = thymine
  modified_base 36: mod_base = OTHER; note = thymine
  modified_base 38: mod_base = OTHER; note = thymine
  modified_base 41: mod_base = OTHER; note = thymine
  misc_feature 1..42: note = Description of Combined DNA/RNA Molecule: Synthetic oligonucleotide
  source 1..42: mol_type = other RNA

SEQ ID NO: 63 - DNA, 23 bp, synthetic construct
  misc_feature 1..23: note = Description of Artificial Sequence: Synthetic oligonucleotide
  source 1..23: mol_type = other DNA
agtaataatacgactcactatag

SEQ ID NO: 64 - DNA, 58 bp, synthetic construct
  misc_feature 1..58: note = Description of Artificial Sequence: Synthetic oligonucleotide
  source 1..58: mol_type = other DNA
taatacgactcactatagggggccactagggacaggatgttttagagctagaaatagc

SEQ ID NO: 65 - DNA, 50 bp, synthetic construct
  misc_feature 1..50: note = Description of Artificial Sequence: Synthetic oligonucleotide
  source 1..50: mol_type = other DNA
gttttagagctagaaatagcaagttaaaataaggctagtccgttatcaac

SEQ ID NO: 66 - DNA, 50 bp, synthetic construct
  misc_feature 1..50: note = Description of Artificial Sequence: Synthetic oligonucleotide
  source 1..50: mol_type = other DNA
aaaaaaagcaccgactcggtgccactttttcaagttgataacggactagc

SEQ ID NO: 67 - DNA, 23 bp, synthetic construct
  misc_feature 1..23: note = Description of Artificial Sequence: Synthetic oligonucleotide
  source 1..23: mol_type = other DNA
aaaaaaagcaccgactcggtgcc

SEQ ID NO: 68 - DNA, 43 bp, synthetic construct
  misc_feature 1..43: note = Description of Artificial Sequence: Synthetic oligonucleotide
  source 1..43: mol_type = other DNA
agtaataatacgactcactatagggggccactagggacaggat

SEQ ID NO: 69 - DNA, 42 bp, synthetic construct; identical to SEQ ID NO: 37
  misc_feature 1..42: note = Description of Artificial Sequence: Synthetic oligonucleotide
  source 1..42: mol_type = other DNA

SEQ ID NO: 70 - DNA, 24 bp, synthetic construct
  misc_feature 1..24: note = Description of Artificial Sequence: Synthetic oligonucleotide
  source 1..24: mol_type = other DNA
caggatgtctcagagctatgctgt

SEQ ID NO: 71 - DNA, 58 bp, synthetic construct
  misc_feature 1..58: note = Description of Artificial Sequence: Synthetic oligonucleotide
  source 1..58: mol_type = other DNA
agtaataatacgactcactatagcaggacagcatagcaagttgagataaggctagtcc

SEQ ID NO: 72 - DNA, 42 bp, synthetic construct
  misc_feature 1..42: note = Description of Artificial Sequence: Synthetic oligonucleotide
  source 1..42: mol_type = other DNA
gcaggacagcatagcaagttgagataaggctagtccgttatc

SEQ ID NO: 73 - DNA, 50 bp, synthetic construct
  misc_feature 1..50: note = Description of Artificial Sequence: Synthetic oligonucleotide
  source 1..50: mol_type = other DNA
aagcaccgactcggtgccactttttcaagttgataacggactagccttat

SEQ ID NO: 74 - DNA, 20 bp, synthetic construct
  misc_feature 1..20: note = Description of Artificial Sequence: Synthetic oligonucleotide
  source 1..20: mol_type = other DNA
aagcaccgactcggtgccac

SEQ ID NO: 75 - DNA, 20 bp, synthetic construct
  misc_feature 1..20: note = Description of Artificial Sequence: Synthetic oligonucleotide
  source 1..20: mol_type = other DNA
ccccgttctcctgtggattc

SEQ ID NO: 76 - DNA, 20 bp, synthetic construct
  misc_feature 1..20: note = Description of Artificial Sequence: Synthetic oligonucleotide
  source 1..20: mol_type = other DNA
atcctctctggctccatcgt

SEQ ID NO: 77 - DNA, 52 bp, synthetic construct
  misc_feature 1..52: note = Description of Artificial Sequence: Synthetic oligonucleotide
  source 1..52: mol_type = other DNA
cactctttccctacacgacgctcttccgatctgtttctcatctgtgcccctc

SEQ ID NO: 78 - DNA, 48 bp, synthetic construct
  misc_feature 1..48: note = Description of Artificial Sequence: Synthetic oligonucleotide
  source 1..48: mol_type = other DNA
ggagttcagacgtgtgctcttccgatctgttgcccaccctagtcattg

SEQ ID NO: 79 - DNA, 52 bp, synthetic construct
  misc_feature 1..52: note = Description of Artificial Sequence: Synthetic oligonucleotide
  source 1..52: mol_type = other DNA
cactctttccctacacgacgctcttccgatctccagatggcacattgtcaga

SEQ ID NO: 80 - DNA, 47 bp, synthetic construct
  misc_feature 1..47: note = Description of Artificial Sequence: Synthetic oligonucleotide
  source 1..47: mol_type = other DNA
ggagttcagacgtgtgctcttccgatctcctagtgactgccgtctgc

SEQ ID NO: 81 - DNA, 52 bp, synthetic construct
  misc_feature 1..52: note = Description of Artificial Sequence: Synthetic oligonucleotide
  source 1..52: mol_type = other DNA
cactctttccctacacgacgctcttccgatctacatgcacacccatgttttg

SEQ ID NO: 82 - DNA, 48 bp, synthetic construct
  misc_feature 1..48: note = Description of Artificial Sequence: Synthetic oligonucleotide
  source 1..48: mol_type = other DNA
ggagttcagacgtgtgctcttccgatctaacatttccaggtgacaggc

SEQ ID NO: 83 - DNA, 52 bp, synthetic construct; identical to SEQ ID NO: 81
  misc_feature 1..52: note = Description of Artificial Sequence: Synthetic oligonucleotide
  source 1..52: mol_type = other DNA

SEQ ID NO: 84 - DNA, 48 bp, synthetic construct; identical to SEQ ID NO: 82
  misc_feature 1..48: note = Description of Artificial Sequence: Synthetic oligonucleotide
  source 1..48: mol_type = other DNA

SEQ ID NO: 85 - DNA, 52 bp, synthetic construct
  misc_feature 1..52: note = Description of Artificial Sequence: Synthetic oligonucleotide
  source 1..52: mol_type = other DNA
cactctttccctacacgacgctcttccgatctacatgaaattcaaggccgaa

SEQ ID NO: 86 - DNA, 48 bp, synthetic construct
  misc_feature 1..48: note = Description of Artificial Sequence: Synthetic oligonucleotide
  source 1..48: mol_type = other DNA
ggagttcagacgtgtgctcttccgatctacctgtctgtgaggtggagg

SEQ ID NO: 87 - DNA, 52 bp, synthetic construct
  misc_feature 1..52: note = Description of Artificial Sequence: Synthetic oligonucleotide
  source 1..52: mol_type = other DNA
cactctttccctacacgacgctcttccgatctgctggtggattatgggaatg

SEQ ID NO: 88 - DNA, 48 bp, synthetic construct
  misc_feature 1..48: note = Description of Artificial Sequence: Synthetic oligonucleotide
  source 1..48: mol_type = other DNA
ggagttcagacgtgtgctcttccgatctagaagacctcatccttgggg

SEQ ID NO: 89 - DNA, 52 bp, synthetic construct
  misc_feature 1..52: note = Description of Artificial Sequence: Synthetic oligonucleotide
  source 1..52: mol_type = other DNA
cactctttccctacacgacgctcttccgatctaagaaaggcaagaagcctgg

SEQ ID NO: 90 - DNA, 48 bp, synthetic construct
  misc_feature 1..48: note = Description of Artificial Sequence: Synthetic oligonucleotide
  source 1..48: mol_type = other DNA
ggagttcagacgtgtgctcttccgatctgctggcctgagacattccta

SEQ ID NO: 91 - DNA, 52 bp, synthetic construct
  misc_feature 1..52: note = Description of Artificial Sequence: Synthetic oligonucleotide
  source 1..52: mol_type = other DNA
cactctttccctacacgacgctcttccgatcttgtgtactctccactgccca

SEQ ID NO: 92 - DNA, 48 bp, synthetic construct
  misc_feature 1..48: note = Description of Artificial Sequence: Synthetic oligonucleotide
  source 1..48: mol_type = other DNA
ggagttcagacgtgtgctcttccgatcttcagaacactcccttttgcc

SEQ ID NO: 93 - DNA, 52 bp, synthetic construct
  misc_feature 1..52: note = Description of Artificial Sequence: Synthetic oligonucleotide
  source 1..52: mol_type = other DNA
cactctttccctacacgacgctcttccgatcttctggcaaggagagagatgg

SEQ ID NO: 94 - DNA, 48 bp, synthetic construct
  misc_feature 1..48: note = Description of Artificial Sequence: Synthetic oligonucleotide
  source 1..48: mol_type = other DNA
ggagttcagacgtgtgctcttccgatcttatattcccagggccggtta

SEQ ID NO: 95 - DNA, 57 bp, synthetic construct
  misc_feature 1..57: note = Description of Artificial Sequence: Synthetic oligonucleotide
  source 1..57: mol_type = other DNA
caagcagaagacggcatacgagattacgtgatgtgactggagttcagacgtgtgctc

SEQ ID NO: 96 - DNA, 57 bp, synthetic construct
  misc_feature 1..57: note = Description of Artificial Sequence: Synthetic oligonucleotide
  source 1..57: mol_type = other DNA
caagcagaagacggcatacgagatattgccgagtgactggagttcagacgtgtgctc

SEQ ID NO: 97 - DNA, 57 bp, synthetic construct
  misc_feature 1..57: note = Description of Artificial Sequence: Synthetic oligonucleotide
  source 1..57: mol_type = other DNA
caagcagaagacggcatacgagatattggtcagtgactggagttcagacgtgtgctc

SEQ ID NO: 98 - DNA, 57 bp, synthetic construct
  misc_feature 1..57: note = Description of Artificial Sequence: Synthetic oligonucleotide
  source 1..57: mol_type = other DNA
caagcagaagacggcatacgagattaaaaatggtgactggagttcagacgtgtgctc

SEQ ID NO: 99 - DNA, 57 bp, synthetic construct
  misc_feature 1..57: note = Description of Artificial Sequence: Synthetic oligonucleotide
  source 1..57: mol_type = other DNA
caagcagaagacggcatacgagatatcactgtgtgactggagttcagacgtgtgctc

SEQ ID NO: 100 - DNA, 57 bp, synthetic construct
  misc_feature 1..57: note = Description of Artificial Sequence: Synthetic oligonucleotide
  source 1..57: mol_type = other DNA
caagcagaagacggcatacgagattatttcacgtgactggagttcagacgtgtgctc

SEQ ID NO: 101 - DNA, 58 bp, synthetic construct
  misc_feature 1..58: note = Description of Artificial Sequence: Synthetic oligonucleotide
  source 1..58: mol_type = other DNA
aatgatacggcgaccaccgagatctacaccgtctaatacactctttccctacacgacg

SEQ ID NO: 102 - DNA, 58 bp, synthetic construct
  misc_feature 1..58: note = Description of Artificial Sequence: Synthetic oligonucleotide
  source 1..58: mol_type = other DNA
aatgatacggcgaccaccgagatctacactctctccgacactctttccctacacgacg

SEQ ID NO: 103 - DNA, 58 bp, synthetic construct
  misc_feature 1..58: note = Description of Artificial Sequence: Synthetic oligonucleotide
  source 1..58: mol_type = other DNA
aatgatacggcgaccaccgagatctacactcgactagacactctttccctacacgacg

SEQ ID NO: 104 - DNA, 58 bp, synthetic construct
  misc_feature 1..58: note = Description of Artificial Sequence: Synthetic oligonucleotide
  source 1..58: mol_type = other DNA
aatgatacggcgaccaccgagatctacacttctagctacactctttccctacacgacg

SEQ ID NO: 105 - DNA, 58 bp, synthetic construct
  misc_feature 1..58: note = Description of Artificial Sequence: Synthetic oligonucleotide
  source 1..58: mol_type = other DNA
aatgatacggcgaccaccgagatctacaccctagagtacactctttccctacacgacg

SEQ ID NO: 106 - DNA, 58 bp, synthetic construct
  misc_feature 1..58: note = Description of Artificial Sequence: Synthetic oligonucleotide
  source 1..58: mol_type = other DNA
aatgatacggcgaccaccgagatctacacctattaagacactctttccctacacgacg

SEQ ID NO: 107 - DNA, 21 bp, synthetic construct
  misc_feature 1..21: note = Description of Artificial Sequence: Synthetic oligonucleotide
  source 1..21: mol_type = other DNA
aaaaccacccttctctctggc

SEQ ID NO: 108 - DNA, 21 bp, synthetic construct
  misc_feature 1..21: note = Description of Artificial Sequence: Synthetic oligonucleotide
  source 1..21: mol_type = other DNA
ggagattggagacacggagag

SEQ ID NO: 109 - DNA, 20 bp, synthetic construct
  misc_feature 1..20: note = Description of Artificial Sequence: Synthetic oligonucleotide
  source 1..20: mol_type = other DNA
aaaggtgccttttgtgggga

SEQ ID NO: 110 - DNA, 21 bp, synthetic construct
  misc_feature 1..21: note = Description of Artificial Sequence: Synthetic oligonucleotide
  source 1..21: mol_type = other DNA
acaatgggaaggacagcttct

SEQ ID NO: 111 - DNA, 20 bp, synthetic construct
  misc_feature 1..20: note = Description of Artificial Sequence: Synthetic oligonucleotide
  source 1..20: mol_type = other DNA
tctccgaacttctgctgagc

SEQ ID NO: 112 - DNA, 20 bp, synthetic construct
  misc_feature 1..20: note = Description of Artificial Sequence: Synthetic oligonucleotide
  source 1..20: mol_type = other DNA
tgactagcaaagcaggaggc

SEQ ID NO: 113 - DNA, 20 bp, synthetic construct
  misc_feature 1..20: note = Description of Artificial Sequence: Synthetic oligonucleotide
  source 1..20: mol_type = other DNA
aagtccttcccatcgctgtg

SEQ ID NO: 114 - DNA, 20 bp, synthetic construct
  misc_feature 1..20: note = Description of Artificial Sequence: Synthetic oligonucleotide
  source 1..20: mol_type = other DNA
gggaatgggaatgtgaggca

SEQ ID NO: 115 - DNA, 20 bp, synthetic construct
  misc_feature 1..20: note = Description of Artificial Sequence: Synthetic oligonucleotide
  source 1..20: mol_type = other DNA
gagtccctgctctcctctga

SEQ ID NO: 116 - DNA, 20 bp, synthetic construct
  misc_feature 1..20: note = Description of Artificial Sequence: Synthetic oligonucleotide
  source 1..20: mol_type = other DNA
agggaataccaaaacggcgt

SEQ ID NO: 117 - DNA, 20 bp, synthetic construct
  misc_feature 1..20: note = Description of Artificial Sequence: Synthetic oligonucleotide
  source 1..20: mol_type = other DNA
gtcagagggacacactgtgg

SEQ ID NO: 118 - DNA, 20 bp, synthetic construct
  misc_feature 1..20: note = Description of Artificial Sequence: Synthetic oligonucleotide
  source 1..20: mol_type = other DNA
aggagggagcaggaaagtga

SEQ ID NO: 119 - DNA, 20 bp, synthetic construct
  misc_feature 1..20: note = Description of Artificial Sequence: Synthetic oligonucleotide
  source 1..20: mol_type = other DNA
ctcctgctccatgtgaccac

SEQ ID NO: 120 - DNA, 20 bp, synthetic construct
  misc_feature 1..20: note = Description of Artificial Sequence: Synthetic oligonucleotide
  source 1..20: mol_type = other DNA
gtagtggcacagtcacagct

SEQ ID NO: 121 - DNA, 20 bp, synthetic construct
  misc_feature 1..20: note = Description of Artificial Sequence: Synthetic oligonucleotide
  source 1..20: mol_type = other DNA
gagttgcagactggagctgt

SEQ ID NO: 122 - DNA, 20 bp, synthetic construct
  misc_feature 1..20: note = Description of Artificial Sequence: Synthetic oligonucleotide
  source 1..20: mol_type = other DNA
ttggaggcaaggcatctctg

SEQ ID NO: 123 - DNA, 20 bp, synthetic construct
  misc_feature 1..20: note = Description of Artificial Sequence: Synthetic oligonucleotide
  source 1..20: mol_type = other DNA
aggactcctgctgagaggag

SEQ ID NO: 124 - DNA, 20 bp, synthetic construct
  misc_feature 1..20: note = Description of Artificial Sequence: Synthetic oligonucleotide
  source 1..20: mol_type = other DNA
ggagaactaaagggcgtgct

SEQ ID NO: 125 - DNA, 20 bp, synthetic construct
  misc_feature 1..20: note = Description of Artificial Sequence: Synthetic oligonucleotide
  source 1..20: mol_type = other DNA
accaccacatgttctgggtg

SEQ ID NO: 126 - DNA, 20 bp, synthetic construct
  misc_feature 1..20: note = Description of Artificial Sequence: Synthetic oligonucleotide
  source 1..20: mol_type = other DNA
gcttcctcttccaggctctg

SEQ ID NO: 127 - RNA, 97 nt, synthetic construct
  modified_base 9: mod_base = OTHER; note = thymine
  misc_feature 1..97: note = Description of Combined DNA/RNA Molecule: Synthetic oligonucleotide
  source 1..97: mol_type = other RNA
ggggccactagggacaggatgttttagagctagaaatagcaagttaaaataaggctagtccgttatcaacttgaaaaagtggcaccgagtcggtgct

SEQ ID NO: 128 - RNA, 97 nt, synthetic construct; identical to SEQ ID NO: 127
  modified_base 9: mod_base = OTHER; note = thymine
  misc_feature 1..97: note = Description of Combined DNA/RNA Molecule: Synthetic oligonucleotide
  source 1..97: mol_type = other RNA

SEQ ID NO: 129 - RNA, 103 nt, synthetic construct
  modified_base 9: mod_base = OTHER; note = thymine
  modified_base 31: mod_base = OTHER; note = thymine
  modified_base 34: mod_base = OTHER; note = thymine
  misc_feature 1..103: note = Description of Combined DNA/RNA Molecule: Synthetic polynucleotide
  source 1..103: mol_type = other RNA
ggggccactagggacaggatgttttagagctgctgaaaagcatagcaagttaaaataaggctagtccgttatcaacttgaaaaagtggcaccgagtcggtgct

SEQ ID NO: 130 - RNA, 105 nt, synthetic construct
  modified_base 9: mod_base = OTHER; note = thymine
  modified_base 31: mod_base = OTHER; note = thymine
  modified_base 33: mod_base = OTHER; note = thymine
  modified_base 36: mod_base = OTHER; note = thymine
  modified_base 45: mod_base = OTHER; note = thymine
  misc_feature 1..105: note = Description of Combined DNA/RNA Molecule: Synthetic polynucleotide
  source 1..105: mol_type = other RNA
ggggccactagggacaggatgttttagagctatgctgaaaagcatagcaagttaaaataaggctagtccgttatcaacttgaaaaagtggcaccgagtcggtgct

SEQ ID NO: 131 - RNA, 105 nt, synthetic construct; identical to SEQ ID NO: 130
  modified_base 9: mod_base = OTHER; note = thymine
  modified_base 31: mod_base = OTHER; note = thymine
  modified_base 33: mod_base = OTHER; note = thymine
  modified_base 36: mod_base = OTHER; note = thymine
  modified_base 45: mod_base = OTHER; note = thymine
  modified_base 102: mod_base = OTHER; note = thymine
  misc_feature 1..105: note = Description of Combined DNA/RNA Molecule: Synthetic polynucleotide
  source 1..105: mol_type = other RNA

SEQ ID NO: 132 - RNA, 105 nt, synthetic construct; identical to SEQ ID NO: 130
  modified_base 9: mod_base = OTHER; note = thymine
  modified_base 31: mod_base = OTHER; note = thymine
  modified_base 33: mod_base = OTHER; note = thymine
  modified_base 36: mod_base = OTHER; note = thymine
  modified_base 45: mod_base = OTHER; note = thymine
  modified_base 102: mod_base = OTHER; note = thymine
  misc_feature 1..105: note = Description of Combined DNA/RNA Molecule: Synthetic polynucleotide
  source 1..105: mol_type = other RNA

SEQ ID NO: 133 - DNA, 36 bp, synthetic construct
  misc_feature 1..36: note = Description of Artificial Sequence: Synthetic oligonucleotide
  source 1..36: mol_type = other DNA
tacttccaatccaatgcaccccgttctcctgtggat

SEQ ID NO: 134 - DNA, 40 bp, synthetic construct
  misc_feature 1..40: note = Description of Artificial Sequence: Synthetic oligonucleotide
  source 1..40: mol_type = other DNA
ttatccacttccaatgttattactccctcccaggatcctc

SEQ ID NO: 135 - RNA, 39 nt, synthetic construct
  modified_base 6: mod_base = OTHER; note = thymine
  modified_base 17: mod_base = OTHER; note = thymine
  modified_base 28: mod_base = OTHER; note = thymine
  modified_base 30: mod_base = OTHER; note = thymine
  modified_base 33: mod_base = OTHER; note = thymine
  modified_base 35: mod_base = OTHER; note = thymine
  modified_base 38: mod_base = OTHER; note = thymine
  misc_feature 1..39: note = Description of Combined DNA/RNA Molecule: Synthetic oligonucleotide
  source 1..39: mol_type = other RNA
gccactagggacaggatgtctcagagctatgctgtcctg

SEQ ID NO: 136 - RNA, 39 nt, synthetic construct; identical to SEQ ID NO: 135
  modified_base 6: mod_base = OTHER; note = thymine
  modified_base 28: mod_base = OTHER; note = thymine
  modified_base 30: mod_base = OTHER; note = thymine
  modified_base 33: mod_base = OTHER; note = thymine
  modified_base 35: mod_base = OTHER; note = thymine
  modified_base 38: mod_base = OTHER; note = thymine
  misc_feature 1..39: note = Description of Combined DNA/RNA Molecule: Synthetic oligonucleotide
  source 1..39: mol_type = other RNA

SEQ ID NO: 137 - RNA, 39 nt, synthetic construct; identical to SEQ ID NO: 135
  modified_base 6: mod_base = OTHER; note = thymine
  modified_base 17: mod_base = OTHER; note = thymine
  modified_base 28: mod_base = OTHER; note = thymine
  modified_base 30: mod_base = OTHER; note = thymine
  modified_base 33: mod_base = OTHER; note = thymine
  modified_base 35: mod_base = OTHER; note = thymine
  modified_base 38: mod_base = OTHER; note = thymine
  misc_feature 1..39: note = Description of Combined DNA/RNA Molecule: Synthetic oligonucleotide
  source 1..39: mol_type = other RNA

SEQ ID NO: 138 - RNA, 56 nt, synthetic construct
  modified_base 31: mod_base = OTHER; note = thymine
  modified_base 33: mod_base = OTHER; note = thymine
  modified_base 35: mod_base = OTHER; note = thymine
  modified_base 38..41: mod_base = OTHER; note = thymine
  modified_base 45: mod_base = OTHER; note = thymine
  modified_base 47: mod_base = OTHER; note = thymine
  modified_base 52: mod_base = OTHER; note = thymine
  misc_feature 1..56: note = Description of Combined DNA/RNA Molecule: Synthetic oligonucleotide
  variation 1..15: note = a, c, t, g, unknown or other
  variation 16..20: note = a, c, u, g, unknown or other
  source 1..56: mol_type = other RNA
nnnnnnnnnnnnnnnnnnnngttttagtactctgtaattttaggtatgaggtagac

SEQ ID NO: 139 - RNA, 56 nt, synthetic construct; identical to SEQ ID NO: 138
  modified_base 31: mod_base = OTHER; note = thymine
  modified_base 33: mod_base = OTHER; note = thymine
  modified_base 35: mod_base = OTHER; note = thymine
  modified_base 38..41: mod_base = OTHER; note = thymine
  modified_base 45: mod_base = OTHER; note = thymine
  modified_base 47: mod_base = OTHER; note = thymine
  modified_base 52: mod_base = OTHER; note = thymine
  misc_feature 1..56: note = Description of Combined DNA/RNA Molecule: Synthetic oligonucleotide
  variation 1..20: note = a, c, t, g, unknown or other
  source 1..56: mol_type = other RNA

SEQ ID NO: 140 - RNA, 56 nt, synthetic construct; identical to SEQ ID NO: 138
  modified_base 35: mod_base = OTHER; note = thymine
  modified_base 38..41: mod_base = OTHER; note = thymine
  modified_base 45: mod_base = OTHER; note = thymine
  modified_base 47: mod_base = OTHER; note = thymine
  modified_base 52: mod_base = OTHER; note = thymine
  misc_feature 1..56: note = Description of Combined DNA/RNA Molecule: Synthetic oligonucleotide
  variation 1..20: note = a, c, t, g, unknown or other
  source 1..56: mol_type = other RNA

SEQ ID NO: 141 - RNA, 56 nt, synthetic construct; identical to SEQ ID NO: 138
  modified_base 28: mod_base = OTHER; note = thymine
  modified_base 31: mod_base = OTHER; note = thymine
  modified_base 33: mod_base = OTHER; note = thymine
  modified_base 35: mod_base = OTHER; note = thymine
  modified_base 38..41: mod_base = OTHER; note = thymine
  modified_base 45: mod_base = OTHER; note = thymine
  modified_base 47: mod_base = OTHER; note = thymine
  modified_base 52: mod_base = OTHER; note = thymine
  misc_feature 1..56: note = Description of Combined DNA/RNA Molecule: Synthetic oligonucleotide
  variation 1..2: note = a, c, t, g, unknown or other
  variation 3..4: note = a, c, u, g, unknown or other
  variation 5..14: note = a, c, t, g, unknown or other
  variation 15..17: note = a, c, u, g, unknown or other
  variation 18: note = a, c, t, g, unknown or other
  variation 19: note = a, c, u, g, unknown or other
  variation 20: note = a, c, t, g, unknown or other
  source 1..56: mol_type = other RNA

SEQ ID NO: 142 - RNA, 85 nt, synthetic construct
  misc_feature 1..85: note = Description of Artificial Sequence: Synthetic oligonucleotide
  source 1..85: mol_type = other RNA
attgtacttatacctaaaattacagaatctactaaaacaaggcaaaatgccgtgtttatctcgtcaacttgttggcgagattttt

SEQ ID NO: 143 - RNA, 106 nt, synthetic construct
  modified_base 31: mod_base = OTHER; note = thymine
  modified_base 33: mod_base = OTHER; note = thymine
  misc_feature 1..106: note = Description of Combined DNA/RNA Molecule: Synthetic polynucleotide
  variation 1..15: note = a, c, t, g, unknown or other
  variation 16..20: note = a, c, u, g, unknown or other
  source 1..106: mol_type = other RNA
nnnnnnnnnnnnnnnnnnnngttttagtactctggaaacagaatctactaaaaacaaggccaaaatgccggtgtttatcttcgtcaactttgttggcgaggatttt

SEQ ID NO: 144 - RNA, 106 nt, synthetic construct; identical to SEQ ID NO: 143
  modified_base 31: mod_base = OTHER; note = thymine
  modified_base 33: mod_base = OTHER; note = thymine
  misc_feature 1..106: note = Description of Combined DNA/RNA Molecule: Synthetic polynucleotide
  variation 1..20: note = a, c, t, g, unknown or other
  source 1..106: mol_type = other RNA

SEQ ID NO: 145 - RNA, 106 nt, synthetic construct; identical to SEQ ID NO: 143
  misc_feature 1..106: note = Description of Combined DNA/RNA Molecule: Synthetic polynucleotide
  variation 1..20: note = a, c, t, g, unknown or other
  source 1..106: mol_type = other RNA

SEQ ID NO: 146 - RNA, 106 nt, synthetic construct; identical to SEQ ID NO: 143
  modified_base 28: mod_base = OTHER; note = thymine
  modified_base 31: mod_base = OTHER; note = thymine
  modified_base 33: mod_base = OTHER; note = thymine
  misc_feature 1..106: note = Description of Combined DNA/RNA Molecule: Synthetic polynucleotide
  variation 1..2: note = a, c, t, g, unknown or other
  variation 3..4: note = a, c, u, g, unknown or other
  variation 5..14: note = a, c, t, g, unknown or other
  variation 15..17: note = a, c, u, g, unknown or other
  variation 18: note = a, c, t, g, unknown or other
  variation 19: note = a, c, u, g, unknown or other
  variation 20: note = a, c, t, g, unknown or other
  source 1..106: mol_type = other RNA

SEQ ID NO: 147 - RNA, 56 nt, synthetic construct
  modified_base 31: mod_base = OTHER; note = thymine
  modified_base 33: mod_base = OTHER; note = thymine
  modified_base 39..41: mod_base = OTHER; note = thymine
  modified_base 45: mod_base = OTHER; note = thymine
  modified_base 49: mod_base = OTHER; note = thymine
  modified_base 51: mod_base = OTHER; note = thymine
  misc_feature 1..56: note = Description of Combined DNA/RNA Molecule: Synthetic oligonucleotide
  variation 1..15: note = a, c, t, g, unknown or other
  variation 16..20: note = a, c, u, g, unknown or other
  source 1..56: mol_type = other RNA
nnnnnnnnnnnnnnnnnnnngtttttgtactctcaagatttaagtaactgtacaac

SEQ ID NO: 148 - RNA, 56 nt, synthetic construct; identical to SEQ ID NO: 147
  modified_base 28: mod_base = OTHER; note = thymine
  modified_base 31: mod_base = OTHER; note = thymine
  modified_base 33: mod_base = OTHER; note = thymine
  modified_base 39..41: mod_base = OTHER; note = thymine
  modified_base 45: mod_base = OTHER; note = thymine
  modified_base 49: mod_base = OTHER; note = thymine
  modified_base 51: mod_base = OTHER; note = thymine
  misc_feature 1..56: note = Description of Combined DNA/RNA Molecule: Synthetic oligonucleotide
  variation 1..20: note = a, c, t, g, unknown or other
  source 1..56: mol_type = other RNA

SEQ ID NO: 149 - RNA, 56 nt, synthetic construct; identical to SEQ ID NO: 147
  modified_base 33: mod_base = OTHER; note = thymine
  modified_base 39..41: mod_base = OTHER; note = thymine
  modified_base 45: mod_base = OTHER; note = thymine
  modified_base 49: mod_base = OTHER; note = thymine
  modified_base 51: mod_base = OTHER; note = thymine
  misc_feature 1..56: note = Description of Combined DNA/RNA Molecule: Synthetic oligonucleotide
  variation 1..20: note = a, c, t, g, unknown or other
  source 1..56: mol_type = other RNA

SEQ ID NO: 150 - RNA, 89 nt, synthetic construct
  misc_feature 1..89: note = Description of Artificial Sequence: Synthetic oligonucleotide
  source 1..89: mol_type = other RNA
cttacacagttacttaaatcttgcagaagctacaaagataaggcttcatgccgaaatcaacaccctgtcattttatggcagggtgtttt

SEQ ID NO: 151 - RNA, 106 nt, synthetic construct
  modified_base 31: mod_base = OTHER; note = thymine
  misc_feature 1..106: note = Description of Combined DNA/RNA Molecule: Synthetic polynucleotide
  variation 1..15: note = a, c, t, g, unknown or other
  variation 16..20: note = a, c, u, g, unknown or other
  source 1..106: mol_type = other RNA
nnnnnnnnnnnnnnnnnnnngtttttgtactcgaaagaagctacaaagattaaggcttcaatgccgaaattcaacacccttgtcattttaatggcagggttgtttt

SEQ ID NO: 152 - RNA, 106 nt, synthetic construct; identical to SEQ ID NO: 151
  modified_base 31: mod_base = OTHER; note = thymine
  misc_feature 1..106: note = Description of Combined DNA/RNA Molecule: Synthetic polynucleotide
  variation 1..20: note = a, c, t, g, unknown or other
  source 1..106: mol_type = other RNA

SEQ ID NO: 153 - RNA, 106 nt, synthetic construct; identical to SEQ ID NO: 151
  misc_feature 1..106: note = Description of Combined DNA/RNA Molecule: Synthetic polynucleotide
  variation 1..20: note = a, c, t, g, unknown or other
  source 1..106: mol_type = other RNA

SEQ ID NO: 154 - RNA, 56 nt, synthetic construct
  modified_base 34..35: mod_base = OTHER; note = thymine
  modified_base 37: mod_base = OTHER; note = thymine
  modified_base 40..42: mod_base = OTHER; note = thymine
  modified_base 48: mod_base = OTHER; note = thymine
  modified_base 51: mod_base = OTHER; note = thymine
  modified_base 56: mod_base = OTHER; note = thymine
  misc_feature 1..56: note = Description of Combined DNA/RNA Molecule: Synthetic oligonucleotide
  variation 1..15: note = a, c, t, g, unknown or other
  variation 16..20: note = a, c, u, g, unknown or other
  source 1..56: mol_type = other RNA
nnnnnnnnnnnnnnnnnnnngttgtagctcccattctcatttcgcagtgctacaat

SEQ ID NO: 155 - RNA, 56 nt, synthetic construct; identical to SEQ ID NO: 154
  modified_base 29: mod_base = OTHER; note = thymine
  modified_base 34..35: mod_base = OTHER; note = thymine
  modified_base 37: mod_base = OTHER; note = thymine
  modified_base 40..42: mod_base = OTHER; note = thymine
  modified_base 48: mod_base = OTHER; note = thymine
  modified_base 51: mod_base = OTHER; note = thymine
  modified_base 56: mod_base = OTHER; note = thymine
  misc_feature 1..56: note = Description of Combined DNA/RNA Molecule: Synthetic oligonucleotide
  variation 1..20: note = a, c, t, g, unknown or other
  source 1..56: mol_type = other RNA

SEQ ID NO: 156 - RNA, 56 nt, synthetic construct; identical to SEQ ID NO: 154
  modified_base 34..35: mod_base = OTHER; note = thymine
  modified_base 37: mod_base = OTHER; note = thymine
  modified_base 40..42: mod_base = OTHER; note = thymine
  modified_base 48: mod_base = OTHER; note = thymine
  modified_base 51: mod_base = OTHER; note = thymine
  modified_base 56: mod_base = OTHER; note = thymine
  misc_feature 1..56: note = Description of Combined DNA/RNA Molecule: Synthetic oligonucleotide
  variation 1..20: note = a, c, t, g, unknown or other
  source 1..56: mol_type = other RNA

SEQ ID NO: 157 - RNA, 119 nt, synthetic construct
  misc_feature 1..119: note = Description of Artificial Sequence: Synthetic polynucleotide
  source 1..119: mol_type = other RNA
attgtcgcactgcgaaatgagaaccgttgctacaataaggccgtctgaaaagatgtgccgcaacgctctgccccttaaagcttctgctttaaggggcatcgtttatttcggttaaaaat

SEQ ID NO: 158 - RNA, 110 nt, synthetic construct
  modified_base 34..35: mod_base = OTHER; note = thymine
  modified_base 37: mod_base = OTHER; note = thymine
  misc_feature 1..110: note = Description of Combined DNA/RNA Molecule: Synthetic polynucleotide
  variation 1..15: note = a, c, t, g, unknown or other
  variation 16..20: note = a, c, u, g, unknown or other
  source 1..110: mol_type = other RNA
nnnnnnnnnnnnnnnnnnnngttgtagctcccattctcgaaagagaaccggttgctacaaataaggccgttctgaaaagaatgtgccgcaaacgctctgcccccttaaag

SEQ ID NO: 159 - RNA, 110 nt, synthetic construct; identical to SEQ ID NO: 158
  modified_base 34..35: mod_base = OTHER; note = thymine
  modified_base 37: mod_base = OTHER; note = thymine
  misc_feature 1..110: note = Description of Combined DNA/RNA Molecule: Synthetic polynucleotide
  variation 1..20: note = a, c, t, g, unknown or other
  source 1..110: mol_type = other RNA

SEQ ID NO: 160 - RNA, 110 nt, synthetic construct; identical to SEQ ID NO: 158
  modified_base 34..35: mod_base = OTHER; note = thymine
  modified_base 37: mod_base = OTHER; note = thymine
  misc_feature 1..110: note = Description of Combined DNA/RNA Molecule: Synthetic polynucleotide
  variation 1..20: note = a, c, t, g, unknown or other
  source 1..110: mol_type = other RNA

SEQ ID NO: 161 - RNA, 56 nt, synthetic construct
  modified_base 31: mod_base = OTHER; note = thymine
  modified_base 33: mod_base = OTHER; note = thymine
  modified_base 39..41: mod_base = OTHER; note = thymine
  modified_base 45: mod_base = OTHER; note = thymine
  modified_base 51: mod_base = OTHER; note = thymine
  misc_feature 1..56: note = Description of Combined DNA/RNA Molecule: Synthetic oligonucleotide
  variation 1..14: note = a, c, t, g, unknown or other
  variation 15..20: note = a, c, u, g, unknown or other
  source 1..56: mol_type = other RNA
nnnnnnnnnnnnnnnnnnnngtttttgtactctcaagatttaagtaaccgtaaaac

SEQ ID NO: 162 - RNA, 56 nt, synthetic construct; identical to SEQ ID NO: 161
  modified_base 28: mod_base = OTHER; note = thymine
  modified_base 31: mod_base = OTHER; note = thymine
  modified_base 33: mod_base = OTHER; note = thymine
  modified_base 39..41: mod_base = OTHER; note = thymine
  modified_base 45: mod_base = OTHER; note = thymine
  modified_base 51: mod_base = OTHER; note = thymine
  misc_feature 1..56: note = Description of Combined DNA/RNA Molecule: Synthetic oligonucleotide
  variation 1..20: note = a, c, t, g, unknown or other
  source 1..56: mol_type = other RNA

SEQ ID NO: 163 - RNA, 56 nt, synthetic construct; identical to SEQ ID NO: 161
  modified_base 39..41: mod_base = OTHER; note = thymine
  modified_base 45: mod_base = OTHER; note = thymine
  modified_base 51: mod_base = OTHER; note = thymine
  misc_feature 1..56: note = Description of Combined DNA/RNA Molecule: Synthetic oligonucleotide
  variation 1..20: note = a, c, t, g, unknown or other
  source 1..56: mol_type = other RNA

SEQ ID NO: 164 - RNA, 90 nt, synthetic construct
  misc_feature 1..90: note = Description of Artificial Sequence: Synthetic oligonucleotide
  source 1..90: mol_type = other RNA
cttgcacggttacttaaatcttgctgagcctacaaagataaggctttatgccgaattcaagcaccccatgttttgacatgaggtgctttt

SEQ ID NO: 165 - RNA, 106 nt, synthetic construct
  modified_base 31: mod_base = OTHER; note = thymine
  misc_feature 1..106: note = Description of Combined DNA/RNA Molecule: Synthetic polynucleotide
  variation 1..15: note = a, c, t, g, unknown or other
  variation 16..20: note = a, c, u, g, unknown or other
  source 1..106: mol_type = other RNA
nnnnnnnnnnnnnnnnnnnngtttttgtactcgaaagagcctacaaagattaaggctttaatgccgaatttcaagcacccccatgttttggacatgaggttgcttt

SEQ ID NO: 166 - RNA, 106 nt, synthetic construct; identical to SEQ ID NO: 165
  modified_base 31: mod_base = OTHER; note = thymine
  misc_feature 1..106: note = Description of Combined DNA/RNA Molecule: Synthetic polynucleotide
  variation 1..20: note = a, c, t, g, unknown or other
  source 1..106: mol_type = other RNA

SEQ ID NO: 167 - RNA, 106 nt, synthetic construct; identical to SEQ ID NO: 165
  modified_base 31: mod_base = OTHER; note = thymine
  misc_feature 1..106: note = Description of Combined DNA/RNA Molecule: Synthetic polynucleotide
  variation 1..20: note = a, c, t, g, unknown or other
  source 1..106: mol_type = other RNA

SEQ ID NO: 168 - RNA, 11 nt, synthetic construct
  misc_feature 1..11: note = Description of Artificial Sequence: Synthetic oligonucleotide
  source 1..11: mol_type = other RNA
aatttctactg

SEQ ID NO: 169 - RNA, 11 nt, synthetic construct
  modified_base 5: mod_base = OTHER; note = thymine
  modified_base 7: mod_base = OTHER; note = thymine
  misc_feature 1..11: note = Description of Combined DNA/RNA Molecule: Synthetic oligonucleotide
  source 1..11: mol_type = other RNA
aatttctactg

SEQ ID NO: 170 - RNA, 11 nt, synthetic construct
  misc_feature 1..11: note = Description of Artificial Sequence: Synthetic oligonucleotide
  source 1..11: mol_type = other RNA
aatttctactg

SEQ ID NO: 171 - RNA, 11 nt, synthetic construct
  modified_base 5: mod_base = OTHER; note = thymine
  modified_base 7: mod_base = OTHER; note = thymine
  misc_feature 1..11: note = Description of Combined DNA/RNA Molecule: Synthetic oligonucleotide
  source 1..11: mol_type = other RNA
aatttctactg

SEQ ID NO: 172-187 - skipped (16 entries)

SEQ ID NO: 188 - RNA, 44 nt, synthetic construct
  modified_base 15: mod_base = OTHER; note = thymine
  misc_feature 1..44: note = Description of Combined DNA/RNA Molecule: Synthetic oligonucleotide
  variation 20..44: note = a, c, u, g, unknown or other
  source 1..44: mol_type = other RNA
aatttctactgttgtagatnnnnnnnnnnnnnnnnnnnnnnnnn

SEQ ID NO: 189 - RNA, 44 nt, synthetic construct; identical to SEQ ID NO: 188
  modified_base 5: mod_base = OTHER; note = thymine
  modified_base 7: mod_base = OTHER; note = thymine
  misc_feature 1..44: note = Description of Combined DNA/RNA Molecule: Synthetic oligonucleotide
  variation 20..44: note = a, c, u, g, unknown or other
  source 1..44: mol_type = other RNA

SEQ ID NO: 190 - RNA, 44 nt, synthetic construct; identical to SEQ ID NO: 188
  modified_base 5: mod_base = OTHER; note = thymine
  modified_base 7: mod_base = OTHER; note = thymine
  modified_base 15: mod_base = OTHER; note = thymine
  misc_feature 1..44: note = Description of Combined DNA/RNA Molecule: Synthetic oligonucleotide
  variation 20..44: note = a, c, u, g, unknown or other
  source 1..44: mol_type = other RNA

SEQ ID NO: 191 - RNA, 44 nt, synthetic construct; identical to SEQ ID NO: 188
  misc_feature 1..44: note = Description of Combined DNA/RNA Molecule: Synthetic oligonucleotide
  variation 20..44: note = a, c, t, g, unknown or other
  source 1..44: mol_type = other RNA

SEQ ID NO: 192 - RNA, 44 nt, synthetic construct; identical to SEQ ID NO: 188
  modified_base 5: mod_base = OTHER; note = thymine
  modified_base 7: mod_base = OTHER; note = thymine
  misc_feature 1..44: note = Description of Combined DNA/RNA Molecule: Synthetic oligonucleotide
  variation 20..44: note = a, c, t, g, unknown or other
  source 1..44: mol_type = other RNA

SEQ ID NO: 193 - RNA, 44 nt, synthetic construct; identical to SEQ ID NO: 188
  modified_base 5: mod_base = OTHER; note = thymine
  modified_base 7: mod_base = OTHER; note = thymine
  misc_feature 1..44: note = Description of Combined DNA/RNA Molecule: Synthetic oligonucleotide
  variation 20..21: note = a, c, u, g, unknown or other
  variation 22..44: note = a, c, t, g, unknown or other
  source 1..44: mol_type = other RNA

SEQ ID NO: 194 - RNA, 44 nt, synthetic construct; identical to SEQ ID NO: 188
  modified_base 5: mod_base = OTHER; note = thymine
  modified_base 7: mod_base = OTHER; note = thymine
  misc_feature 1..44: note = Description of Combined DNA/RNA Molecule: Synthetic oligonucleotide
  variation 20..24: note = a, c, u, g, unknown or other
  variation 25..44: note = a, c, t, g, unknown or other
  source 1..44: mol_type = other RNA

SEQ ID NO: 195 - RNA, 44 nt, synthetic construct; identical to SEQ ID NO: 188
  modified_base 5: mod_base = OTHER; note = thymine
  modified_base 7: mod_base = OTHER; note = thymine
  misc_feature 1..44: note = Description of Combined DNA/RNA Molecule: Synthetic oligonucleotide
  variation 20..29: note = a, c, u, g, unknown or other
  variation 30..44: note = a, c, t, g, unknown or other
  source 1..44: mol_type = other RNA

SEQ ID NO: 196 - RNA, 44 nt, synthetic construct; identical to SEQ ID NO: 188
  modified_base 15: mod_base = OTHER; note = thymine
  misc_feature 1..44: note = Description of Combined DNA/RNA Molecule: Synthetic oligonucleotide
  variation 20..44: note = a, c, t, g, unknown or other
  source 1..44: mol_type = other RNA

SEQ ID NO: 197 - RNA, 44 nt, synthetic construct; identical to SEQ ID NO: 188
  modified_base 15: mod_base = OTHER; note = thymine
  misc_feature 1..44: note = Description of Artificial Sequence: Synthetic oligonucleotide
  misc_feature 1..44: note = Description of Combined DNA/RNA Molecule: Synthetic oligonucleotide
  variation 20..21: note = a, c, u, g, unknown or other
  variation 22..44: note = a, c, t, g, unknown or other
  source 1..44: mol_type = other RNA

SEQ ID NO: 198 - RNA, 44 nt, synthetic construct; identical to SEQ ID NO: 188
  modified_base 15: mod_base = OTHER; note = thymine
  misc_feature 1..44: note = Description of Combined DNA/RNA Molecule: Synthetic oligonucleotide
  variation 20..24: note = a, c, u, g, unknown or other
  variation 25..44: note = a, c, t, g, unknown or other
  source 1..44: mol_type = other RNA

SEQ ID NO: 199 - RNA, 44 nt, synthetic construct; identical to SEQ ID NO: 188
  modified_base 15: mod_base = OTHER; note = thymine
  misc_feature 1..44: note = Description of Combined DNA/RNA Molecule: Synthetic oligonucleotide
  variation 20..29: note = a, c, u, g, unknown or other
  variation 30..44: note = a, c, t, g, unknown or other
  source 1..44: mol_type = other RNA

SEQ ID NO: 200 - RNA, 44 nt, synthetic construct; identical to SEQ ID NO: 188
  modified_base 5: mod_base = OTHER; note = thymine
  modified_base 7: mod_base = OTHER; note = thymine
  modified_base 15: mod_base = OTHER; note = thymine
  misc_feature 1..44: note = Description of Combined DNA/RNA Molecule: Synthetic oligonucleotide
  variation 20..44: note = a, c, t, g, unknown or other
  source 1..44: mol_type = other RNA

SEQ ID NO: 201 - RNA, 44 nt, synthetic construct; identical to SEQ ID NO: 188
  modified_base 5: mod_base = OTHER; note = thymine
  modified_base 7: mod_base = OTHER; note = thymine
  modified_base 15: mod_base = OTHER; note = thymine
  misc_feature 1..44: note = Description of Combined DNA/RNA Molecule: Synthetic oligonucleotide
  variation 20..21: note = a, c, u, g, unknown or other
  variation 22..44: note = a, c, t, g, unknown or other
  source 1..44: mol_type = other RNA

SEQ ID NO: 202 - RNA, 44 nt, synthetic construct; identical to SEQ ID NO: 188
  modified_base 5: mod_base = OTHER; note = thymine
  modified_base 7: mod_base = OTHER; note = thymine
  modified_base 15: mod_base = OTHER; note = thymine
  misc_feature 1..44: note = Description of Combined DNA/RNA Molecule: Synthetic oligonucleotide
  variation 20..24: note = a, c, u, g, unknown or other
  variation 25..44: note = a, c, t, g, unknown or other
  source 1..44: mol_type = other RNA

SEQ ID NO: 203 - RNA, 44 nt, synthetic construct; identical to SEQ ID NO: 188
  modified_base 5: mod_base = OTHER; note = thymine
  modified_base 7: mod_base = OTHER; note = thymine
  modified_base 15: mod_base = OTHER; note = thymine
  misc_feature 1..44: note = Description of Combined DNA/RNA Molecule: Synthetic oligonucleotide
  variation 20..29: note = a, c, u, g, unknown or other
  variation 30..44: note = a, c, t, g, unknown or other
  source 1..44: mol_type = other RNA

SEQ ID NO: 204 - RNA, 97 nt, synthetic construct
  modified_base 1: mod_base = OTHER; note = thymine
  modified_base 7: mod_base = OTHER; note = thymine
  modified_base 13: mod_base = OTHER; note = thymine
  misc_feature 1..97: note = Description of Combined DNA/RNA Molecule: Synthetic polynucleotide
  source 1..97: mol_type = other RNA
tacgcgtacgcgtacgtgtggttttagagctagaaatagcaagttaaaataaggctagtccgttatcaacttgaaaaagtggcaccgagtcggtgct

SEQ ID NO: 205 - RNA, 105 nt, synthetic construct
  modified_base 1: mod_base = OTHER; note = thymine
  modified_base 7: mod_base = OTHER; note = thymine
  modified_base 13: mod_base = OTHER; note = thymine
  modified_base 31: mod_base = OTHER; note = thymine
  modified_base 33: mod_base = OTHER; note = thymine
  modified_base 36: mod_base = OTHER; note = thymine
  modified_base 45: mod_base = OTHER; note = thymine
  misc_feature 1..105: note = Description of Combined DNA/RNA Molecule: Synthetic polynucleotide
  source 1..105: mol_type = other RNA
tacgcgtacgcgtacgtgtggttttagagctatgctgaaaagcatagcaagttaaaataaggctagtccgttatcaacttgaaaaagtggcaccgagtcggtgct

SEQ ID NO: 206 - RNA, 105 nt, synthetic construct; identical to SEQ ID NO: 205
  modified_base 1: mod_base = OTHER; note = thymine
  modified_base 7: mod_base = OTHER; note = thymine
  modified_base 13: mod_base = OTHER; note = thymine
  modified_base 31: mod_base = OTHER; note = thymine
  modified_base 33: mod_base = OTHER; note = thymine
  modified_base 36: mod_base = OTHER; note = thymine
  modified_base 45: mod_base = OTHER; note = thymine
  modified_base 102: mod_base = OTHER; note = thymine
  misc_feature 1..105: note = Description of Combined DNA/RNA Molecule: Synthetic polynucleotide
  source 1..105: mol_type = other RNA

SEQ ID NO: 207 - RNA, 98 nt, synthetic construct
  misc_feature 1..98: note = Description of Artificial Sequence: Synthetic oligonucleotide
  source 1..98: mol_type = other RNA
ggcgtacgcgtacgtgtggttttagagctagaaatagcaagttaaaataaggctagtccgttatcaacttgaaaaagtggcaccgagtcggtgctttt

SEQ ID NO: 208 - DNA, 60 bp, synthetic construct
  misc_feature 1..60: note = Description of Artificial Sequence: Synthetic oligonucleotide
  source 1..60: mol_type = other DNA
ctacactctttccctacacgacgctcttccgatctaaggcgcaaatgagtagcagcgcac

SEQ ID NO: 209 - DNA, 57 bp, synthetic construct
  misc_feature 1..57: note = Description of Artificial Sequence: Synthetic oligonucleotide
  source 1..57: mol_type = other DNA
caagcagaagacggcatacgagctcttccgatctcacctgctgggaattgtaccgta

SEQ ID NO: 210 - DNA, 60 bp, synthetic construct
  misc_feature 1..60: note = Description of Artificial Sequence: Synthetic oligonucleotide
  source 1..60: mol_type = other DNA
ctacactctttccctacacgacgctcttccgatctggaacgcaaatgagtagcagcgcac

SEQ ID NO: 211 - DNA, 60 bp, synthetic construct
  misc_feature 1..60: note = Description of Artificial Sequence: Synthetic oligonucleotide
  source 1..60: mol_type = other DNA
ctacactctttccctacacgacgctcttccgatctccttcgcaaatgagtagcagcgcac

SEQ ID NO: 212 - DNA, 60 bp, synthetic construct
  misc_feature 1..60: note = Description of Artificial Sequence: Synthetic oligonucleotide
  source 1..60: mol_type = other DNA
ctacactctttccctacacgacgctcttccgatctgaagcgcaaatgagtagcagcgcac

SEQ ID NO: 213 - DNA, 60 bp, synthetic construct
  misc_feature 1..60: note = Description of Artificial Sequence: Synthetic oligonucleotide
  source 1..60: mol_type = other DNA
ctacactctttccctacacgacgctcttccgatctaggacgcaaatgagtagcagcgcac

SEQ ID NO: 214 - DNA, 43 bp, synthetic construct
  misc_feature 1..43: note = Description of Artificial Sequence: Synthetic oligonucleotide
  source 1..43: mol_type = other DNA
aatgatacggcgaccaccgagatctacactctttccctacacg

SEQ ID NO: 215 - DNA, 18 bp, synthetic construct
  misc_feature 1..18: note = Description of Artificial Sequence: Synthetic oligonucleotide
  source 1..18: mol_type = other DNA
caagcagaagacggcata

SEQ ID NO: 216 - DNA, 56 bp, Zea mays
  source 1..56: mol_type = genomic DNA
cagcgcacgtatatatacgcgtacgcgtacgtgtgaggtatatatatcctccgccg

SEQ ID NO: 217 - DNA, 55 bp, Zea mays
  source 1..55: mol_type = genomic DNA
cagcgcacgtatatatacgcgtacgcgtacgttgaggtatatatatcctccgccg

SEQ ID NO: 218 - DNA, 57 bp, Zea mays
  source 1..57: mol_type = genomic DNA
cagcgcacgtatatatacgcgtacgcgtacgttgtgaggtatatatatcctccgccg

SEQ ID NO: 219 - DNA, 55 bp, Zea mays
  source 1..55: mol_type = genomic DNA
cagcgcacgtatatatacgcgtacgcgtacggtgaggtatatatatcctccgccg

SEQ ID NO: 220 - DNA, 27 bp, Zea mays
  source 1..27: mol_type = genomic DNA
cagcgcacgtatatatatcctccgccg

SEQ ID NO: 221 - DNA, 55 bp, Zea mays; identical to SEQ ID NO: 217
  source 1..55: mol_type = genomic DNA

SEQ ID NO: 222 - DNA, 52 bp, Zea mays
  source 1..52: mol_type = genomic DNA
cagcgcacgtatatatacgcgtacgcgtatgaggtatatatatcctccgccg

SEQ ID NO: 223 - DNA, 55 bp, Zea mays; identical to SEQ ID NO: 217
  source 1..55: mol_type = genomic DNA

SEQ ID NO: 224 - RNA, 97 nt, synthetic construct
  modified_base 9: mod_base = OTHER; note = thymine
  modified_base 14: mod_base = OTHER; note = thymine
  misc_feature 1..97: note = Description of Combined DNA/RNA Molecule: Synthetic oligonucleotide
  source 1..97: mol_type = other RNA
ggccgaggtcgactaccggcgttttagagctagaaatagcaagttaaaataaggctagtccgttatcaacttgaaaaagtggcaccgagtcggtgct

SEQ ID NO: 225 - RNA, 105 nt, synthetic construct
  modified_base 9: mod_base = OTHER; note = thymine
  modified_base 14: mod_base = OTHER; note = thymine
  modified_base 31: mod_base = OTHER; note = thymine
  modified_base 33: mod_base = OTHER; note = thymine
  modified_base 36: mod_base = OTHER; note = thymine
  modified_base 45: mod_base = OTHER; note = thymine
  misc_feature 1..105: note = Description of Combined DNA/RNA Molecule: Synthetic polynucleotide
  source 1..105: mol_type = other RNA
ggccgaggtcgactaccggcgttttagagctatgctgaaaagcatagcaagttaaaataaggctagtccgttatcaacttgaaaaagtggcaccgagtcggtgct

SEQ ID NO: 226 - RNA, 105 nt, synthetic construct; identical to SEQ ID NO: 225
  modified_base 9: mod_base = OTHER; note = thymine
  modified_base 14: mod_base = OTHER; note = thymine
  modified_base 31: mod_base = OTHER; note = thymine
  modified_base 33: mod_base = OTHER; note = thymine
  modified_base 36: mod_base = OTHER; note = thymine
  modified_base 45: mod_base = OTHER; note = thymine
  modified_base 102: mod_base = OTHER; note = thymine
  misc_feature 1..105: note = Description of Combined DNA/RNA Molecule: Synthetic polynucleotide
  source 1..105: mol_type = other RNA

SEQ ID NO: 227 - RNA, 124 nt, synthetic construct
  misc_feature 1..124: note = Description of Artificial Sequence: Synthetic polynucleotide
  source 1..124: mol_type = other RNA
gggccgaggtcgactaccggcgttttagagctatgctgttttggaaacaaaacagcatagcaagttaaaataaggctagtccgttatcaacttgaaaaagtggcaccgagtcggtgcttttttt

SEQ ID NO: 228 - DNA, 54 bp, synthetic construct
  misc_feature 1..54: note = Description of Artificial Sequence: Synthetic oligonucleotide
  source 1..54: mol_type = other DNA
caagcagaagacggcatacgagctcttccgatctgccggctggcattgtctctg

SEQ ID NO: 229 - DNA, 58 bp, synthetic construct
  misc_feature 1..58: note = Description of Artificial Sequence: Synthetic oligonucleotide
  source 1..58: mol_type = other DNA
ctacactctttccctacacgacgctcttccgatctttccggacccgttcggcctcagt

SEQ ID NO: 230 - DNA, 58 bp, synthetic construct
  misc_feature 1..58: note = Description of Artificial Sequence: Synthetic oligonucleotide
  source 1..58: mol_type = other DNA
ctacactctttccctacacgacgctcttccgatctggaaggacccgttcggcctcagt

SEQ ID NO: 231 - DNA, 58 bp, synthetic construct
  misc_feature 1..58: note = Description of Artificial Sequence: Synthetic oligonucleotide
  source 1..58: mol_type = other DNA
ctacactctttccctacacgacgctcttccgatctccttggacccgttcggcctcagt

SEQ ID NO: 232 - DNA, 58 bp, synthetic construct
  misc_feature 1..58: note = Description of Artificial Sequence: Synthetic oligonucleotide
  source 1..58: mol_type = other DNA
ctacactctttccctacacgacgctcttccgatcttcctggacccgttcggcctcagt

SEQ ID NO: 233 - DNA, 58 bp, synthetic construct
  misc_feature 1..58: note = Description of Artificial Sequence: Synthetic oligonucleotide
  source 1..58: mol_type = other DNA
ctacactctttccctacacgacgctcttccgatctaaggggacccgttcggcctcagt

SEQ ID NO: 234 - DNA, 39 bp, Zea mays
  source 1..39: mol_type = genomic DNA
agtccgctggccgaggtcgactaccggccggtgaagcac

SEQ ID NO: 235 - DNA, 40 bp, Zea mays
  source 1..40: mol_type = genomic DNA
agtccgctggccgaggtcgactaccaggccggtgaagcac

SEQ ID NO: 236 - DNA, 40 bp, Zea mays
  source 1..40: mol_type = genomic DNA
agtccgctggccgaggtcgacttgccggccggtgaagcac

SEQ ID NO: 237 - DNA, 22 bp, Zea mays
  source 1..22: mol_type = genomic DNA
agtccgctggccggtgaagcac

SEQ ID NO: 238 - DNA, 37 bp, Zea mays
  source 1..37: mol_type = genomic DNA
agtccgctggccgaggtcgaccaggccggtgaagcac

SEQ ID NO: 239 - DNA, 40 bp, Zea mays
  source 1..40: mol_type = genomic DNA
agtccgctggccgaggtcgactacctggccggtgaagcac

SEQ ID NO: 240 - DNA, 18 bp, Zea mays
  source 1..18: mol_type = genomic DNA
agtccgccagtgaagcac

SEQ ID NO: 241 - DNA, 38 bp, Zea mays
  source 1..38: mol_type = genomic DNA
agtccgctggccgaggtcgactacggccggtgaagcac

SEQ ID NO: 242 - DNA, 40 bp, Zea mays
  source 1..40: mol_type = genomic DNA
agtccgctggccgaggtcgactacccggccggtgaagcac

SEQ ID NO: 243 - DNA, 40 bp, Zea mays; identical to SEQ ID NO: 235
  source 1..40: mol_type = genomic DNA

SEQ ID NO: 244 - DNA, 22 bp, Zea mays
  source 1..22: mol_type = genomic DNA
agtccgctggccggtgaagcac

SEQ ID NO: 245 - DNA, 38 bp, Zea mays; identical to SEQ ID NO: 241
  source 1..38: mol_type = genomic DNA

SEQ ID NO: 246 - DNA, 37 bp, Zea mays
  source 1..37: mol_type = genomic DNA
agtccgctggccgaggtcgacttggccggtgaagcac

SEQ ID NO: 247 - DNA, 40 bp, Zea mays; identical to SEQ ID NO: 235
  source 1..40: mol_type = genomic DNA

SEQ ID NO: 248 - DNA, 38 bp, Zea mays; identical to SEQ ID NO: 241
  source 1..38: mol_type = genomic DNA

SEQ ID NO: 249 - DNA, 40 bp, Zea mays; identical to SEQ ID NO: 239
  source 1..40: mol_type = genomic DNA

SEQ ID NO: 250 - DNA, 40 bp, Zea mays; identical to SEQ ID NO: 242
  source 1..40: mol_type = genomic DNA

SEQ ID NO: 251 - DNA, 28 bp, Zea mays
  source 1..28: mol_type = genomic DNA
agtccgctggtcaaggccggcgaagcac

SEQ ID NO: 252 - DNA, 22 bp, Zea mays
  source 1..22: mol_type = genomic DNA
agtccgctggccggtgaagcac

SEQ ID NO: 253 - DNA, 37 bp, Zea mays
  source 1..37: mol_type = genomic DNA
agtccgctggccgaggtcgactaagccggtgaagcac

SEQ ID NO: 254 - DNA, 24 bp, Zea mays
  source 1..24: mol_type = genomic DNA
agtccgctggccgaggtgaagcac